European Patent Application EP 4 656 205 A1, published December 3, 2025. Title: イヌのＢ細胞リンパ腫の治療方法. Applicant: 日本全薬工業株式会社. Application JP. The sequence listing filed with the application follows.

SEQUENCE LISTING (11 sequences)

SEQ ID NO: 1 - protein, 137 aa, Mus musculus
MKLRLSLIFICALLKDVQCEVQLVESGGGLVQPGASLKLSCVASGFTFNDYWMSWVRQTPGKTMEWIGDIKYDGSYTNYAPSLKNRFTISRDNAKSTLYLQMSNVRSEDTATYYCTREAYYYSGDYWGQGVMVTVSS

SEQ ID NO: 2 - protein, 133 aa, Mus musculus
MKTDTLLLWALLLWVPGCTGDIVLTQSPALAVSLGQRATISCKTNQNVDYYGNSYMHWYQQKPGQQPKLLIYLASNLASGIPARFSGRGSGTDFTLTIDPVEADDTATYYCQQSRNLPYTFGAGTKLELKRND

SEQ ID NO: 3 - protein, 110 aa, Canis lupus familiaris
RNDAQPAVYLFQPSPDQLHTGSASVVCLLNSFYPKDINVKWKVDGVIQDTGIQESVTEQDKDSTYSLSSTLTMSSTEYLSHELYSCEITHKSLPSTLIKSFQRSECQRVD

SEQ ID NO: 4 - protein, 334 aa, Canis lupus familiaris
STTAPSVFPLAPSCGSTSGSTVALACLVSGYFPEPVTVSWNSGSLTSGVHTFPSVLQSSGLYSLSSMVTVPSSRWPSETFTCNVAHPASKTKVDKPVPKRENGRVPRPPDCPKCPAPEMLGGPSVFIFPPKPKDTLLIARTPEVTCVVVDLDPEDPEVQISWFVDGKQMQTAKTQPREEQFNGTYRVVSVLPIGHQDWLKGKQFTCKVNNKALPSPIERTISKARGQAHQPSVYVLPPSREELSKNTVSLTCLIKDFFPPDIDVEWQSNGQQEPESKYRTTPPQLDEDGSYFLYSKLSVDKSRWQRGDTFICAVMHEALHNHYTQESLSHSPGK

SEQ ID NO: 5 - protein, 332 aa, Canis lupus familiaris
STTAPSVFPLAPSCGSQSGSTVALACLVSGYIPEPVTVSWNSGSLTSGVHTFPSVLQSSGLYSLSSMVTVPSSRWPSETFTCNVAHPATNTKVDKPVVKECECKCNCNNCPCPGCGLLGGPSVFIFPPKPKDILVTARTPTVTCVVVDLDPENPEVQISWFVDSKQVQTANTQPREEQSNGTYRVVSVLPIGHQDWLSGKQFKCKVNNKALPSPIEEIISKTPGQAHQPNVYVLPPSRDEMSKNTVTLTCLVKDFFPPEIDVEWQSNGQQEPESKYRMTPPQLDEDGSYFLYSKLSVDKSRWQRGDTFICAVMHEALHNHYTQKSLSHSPGK

SEQ ID NO: 6 - protein, 10 aa, synthetic construct
GFTFNDYWMS

SEQ ID NO: 7 - protein, 17 aa, synthetic construct
DIKYDGSYTNYAPSLKN

SEQ ID NO: 8 - protein, 9 aa, synthetic construct
EAYYYSGDY

SEQ ID NO: 9 - protein, 15 aa, synthetic construct
KTNQNVDYYGNSYMH

SEQ ID NO: 10 - protein, 7 aa, synthetic construct
LASNLAS

SEQ ID NO: 11 - protein, 9 aa, synthetic construct
QQSRNLPYT